European Patent Application EP 4 116 408 A1, published January 11, 2023. Title: Method for methanol free culturing of methylotrophic yeast for the biosynthesis of added value products. Applicant: Bioboost Synbio Consulting Inc. The sequence listing filed with the application follows.

SEQUENCE LISTING (21 sequences)

SEQ ID NO: 1 - DNA, 1032 bp, Pichia pastoris
attctggcccttgcacctgatcgcgaaggtggaaatggcagaaggatcagcctggacgaagcaaccagttccaactgctaagtaaagaagatgctagacgaaggagacttcagaggtgaaaagtttgcaagaagagagctgcgggaaataaattttcaatttaaggacttgagtgcgtccatattcgtgtacgtgtccaactgttttccattacctaagaaaaacataaagattaaaaagataaacccaatcgggaaactttagcgtgccgtttcggattccgaaaaacttttggagcgccagatgactatggaaagaggagtgtaccaaaatggcaagtcgggggctactcaccggatagccaatacattctctaggaaccagggatgaatccaggtttttgttgtcacggtaggtcaagcattcacttcttaggaatatctcgttgaaagctacttgaaatcccattgggtgcggaaccagcttctaattaaatagttcgatgatgttctctaagtgggactctacggctcaaacttctacacagcatcatcttagtagtcccttcccaaaacaccattctaggtttcggaacgtaacgaaacaatgttcctctcttcacattgggccgttactctagccttccgaagaaccaataaaagggaccggctgaaacgggtgtggaaactcctgtccagtttatggcaaaggctacagaaatcccaatcttgtcgggatgttgctcctcccaaacgccatattgtactgcagttggtgcgcattttagggaaaatttaccccagatgtcctgattttcgagggctacccccaactccctgtgcttatacttagtctaattctattcagtgtgctgacctacacgtaatgatgtcgtaacccagttaaatggccgaaaaactatttaagtaagtttatttctcctccagatgagactctccttcttttctccgctagttatcaaactataaacctattttacctcaaatacctccaacatcacccacttaaaca

SEQ ID NO: 2 - DNA, 1542 bp, Pichia pastoris
ttattttttgaccgaattctttttttcagaccatatgaccggtccatcttctacggggggattatctatgctttgacctctatcttgattcttttatgattcaaatcacttttacgttatttattacttactggttatttacttagcgccttttctgaaaaacatttactaaaaatcatacatcggcactctcaaacacgacagattgtgatcaagaagcagagacaatcaccactaaggttgcacatttgagccagtaggctcctaatagaggttcgatacttattttgataatacgacatattgtcttacctctgaatgtgtcaatactctctcgttcttcgtctcgtcagctaaaaatataacacttcgagtaagatacgcccaattgaaggctacgagataccagactatcactagtagaactttgacatctgctaaagcagatcaaatatccatttatccagaatcaattaccttcctttagcttgtcgaaggcatgaaaaagctacatgaaaatccccatccttgaagttttgtcagcttaaaggactccatttcctaaaatttcaagcagtcctctcaactaaatttttttccattcctctgcacccagccctcttcatcaaccgtccagccttctcaaaagtccaatgtaagtagcctgcaaattcaggttacaacccctcaattttccatccaagggcgatccttacaaagttaatatcgaacagcagagactaagcgagtcatcatcaccacccaacgatggtgaaaaactttaagcatagattgatggagggtgtatggcacttggcggctgcattagagtttgaaactatggggtaatacatcacatccggaactgatccgactccgagatcatatgcaaagcacgtgatgtaccccgtaaactgctcggattatcgttgcaattcatcgtcttaaacagtacaagaaactttattcatgggtcattggactctgatgaggggcacatttccccaatgattttttgggaaagaaagccgtaagaggacagttaagcgaaagagacaagacaacgaacagcaaaagtgacagctgtcagctacctagtggacagttgggagtttccaattggttggttttgaatttttacccatgttgagttgtccttgcttctccttgcaaacaatgcaagttgataagacatcaccttccaagataggctatttttgtcgcataaatttttgtctcggagtgaaaaccccttttatgtgaacagattacagaagcgtcctacccttcaccggttgagatggggagaaaattaagcgatgaggagacgattattggtataaaagaagcaaccaaaatcccttattgtccttttctgatcagcatcaaagaatattgtcttaaaacgggcttttaactacattgttcttacacattgcaaacctcttccttctatttcggatcaactgtattgactacattgatcttttttaacgaagtttacgacttactaaatccccacaaacaaatcaactgagaaaa

SEQ ID NO: 3 - DNA, 1032 bp, Pichia pastoris; identical to SEQ ID NO: 1

SEQ ID NO: 4 - DNA, 560 bp, Pichia pastoris
atcttcattgatgaaacgttgtgatcggtgtgacttttatagtaaaagctacaactgtttgaaataccaagatatcattgtgaatggctcaaaagggtaatacatctgaaaaacctgaagtgtggaaaattccgatggagccaactcatgataacgcagaagtcccattttgccatcttctcttggtatgaaacggtagaaaatgatccgagtatgccaattgatactcttgattcatgccctatagtttgcgtagggtttaattgatctcctggtctatcgatctgggacgcaatgtagaccccattagtggaaacactgaaagggatccaacactctaggcggacccgctcacagtcatttcaggacaatcaccacaggaatcaactacttctcccagtcttccttgcgtgaagcttcaagcctacaacataacacttcttacttaatctttgattctcgaattgtttacccaatcttgacaacttagcctaagcaatactctggggttatatatagcaattgctcttcctcgctgtagcgttcattccatctttcta

SEQ ID NO: 5 - DNA, 609 bp, Pichia pastoris
tgtcatctgctgatgctgtgagggagaaagaagtaggggtgatacatggtttataggcaaagcatgtttgtttcagatcaaagattagcgtttcaaagttgtggaaaagtgaccatgcaacaatatgcaacacattcggattatctgataagtttcaaagctactaagtaagcccgtttcaagtctccagaccgacatctgccatccagtgattttcttagtcctgaaaaatacgatgtgtaaacataaaccacaaagatcggcctccgaggttgaacccttacgaaagagacatctggtagcgccaatgccaaaaaaaaatcacaccagaaggacaattcccttcccccccagcccattaaagcttaccatttcctattccaatacgttccatagagggcatcgctcggctcattttcgcgtgggtcatactagagcggctagctagtcggctgtttgagctctctaatcgaggggtaaggatgtctaatatgtcataatggctcactatataaagaacccgcttgctcaaccttcgactcctttcccgatcctttgcttgttgcttcttcttttataacaggaaacaaaggaatttatacactttaa

SEQ ID NO: 6 - DNA, 704 bp, Pichia pastoris
aaattaatccataagataaggcaaatgtgcttaagtaattgaaaacagtgttgtgattatataagcatggtatttgaatagaactactggggttaacttatctagtaggatggaagttgagggagatcaagatgcttaaagaaaaggattggccaatatgaaagccataattagcaatacttatttaatcagataattgtggggcattgtgacttgacttttaccaggacttcaaacctcaaccatttaaacagttatagaagacgtaccgtcacttttgcttttaatgtgatctaaatgtgatcacatgaactcaaactaaaatgatatcttttactggacaaaaatgttatcctgcaaacagaaagctttcttctattctaagaagaacatttacattggtgggaaacctgaaaacagaaaataaatactccccagtgaccctatgagcaggatttttgcatccctattgtaggcctttcaaactcacacctaatatttcccgccactcacactatcaatgatcacttcccagttctcttcttcccctattcgtaccatgcaacccttacacgccttttccatttcggttcggatgcgacttccagtctgtggggtacgtagcctattctcttagccggtatttaaacatacaaattcacccaaattctaccttgataaggtaattgattaatttcataaat

SEQ ID NO: 7 - DNA, 501 bp, Pichia pastoris
tccaaaccaaacggtctagcaaaaacgataactttaaagaacttttcaattggttttgtacactaccaccggtttactacctctgccttcggttcttctcctcacatttttcgcaactgggatagcgtagcctaaagtgtcacatgctcgctgctcacattccctacacaacagagattgtcagcagaggaaattgagctccaccattcaacacttgtggatttatgatagtctgtgctatcagctctcttttttttgttgctgtagaatttaccgtgctagcaaccttttaaactttgtttagctctccttccctcttccattcatctgtttcggtccgatccgtctctggtcatctcctccgcattttttttttaccgttagcgataggggtcagatcaattcaatcagttttggcaagggtatttaaaggtggcgaaatccccctccgtttgttgaacacatccaactattctcaacccaaccatctaactaatcgta

SEQ ID NO: 8 - DNA, 1212 bp, Pichia pastoris
cgcagcgttttctgacggtactagaggactcttaggggaaggtagaatcaataaagatcatattaggtaagcaaattttggatggaataggagactaggtgtggatgcgcgatctcgccaaattgcacgaccagagtggatgccggatggtggtaaaccgtttcttcctttttaccacccaagtgcgagtgaaacaccccatggctgctctccgattgcccctctacaggcataagggtgtgactttgtgggcttgaattttacaccccctccaacttttctcgcatcaattgatcctgttaccaatattgcatgcccggaggagacttgccccctaatttcgcggcgtcgtcccggatcgcagggtgagactgtagagaccccacatagtgacaatgattatgtaagaagaggggggtgattcggccggctatcgaactctaacaactaggggggtgaacaatgcccagcagtcctccccactctttgacaaatcagtatcaccgattaacaccccaaatcttattctcaacggtccctcatccttgcacccctctttggacaaatggcagttagcattggtgcactgactgactgcccaaccttaaacccaaatttcttagaaggggcccatctagttagcgaggggtgaaaaattcctccatcggagatgtattgaccgtaagttgctgcttaaaaaaaatcagttcagatagcgagacttttttgatttcgcaacgggagtgcctgttccattcgattgcaattctcaccccttctgcccagtcctgccaattgcccatgaatctgctaatttcgttgattcccacccccctttccaactccacaaattgtccaatctcgttttccatttgggagaatctgcatgtcgactacataaagcgaccggtgtccgaaaagatctgtgtagttttcaacattttgtgctccccccgctgtttgaaaacgggggtgagcgctctccggggtgcgaattcgtgcccaattcctttcaccctgcctattgtagacgtcaacccgcatctggtgcgaatatagcgcacccccaatgatcacaccaacaattggtccacccctccccaatctctaatattcacaattcacctcactataaatacccctgtcctgctcccaaattcttttttccttcttccatcagctactagcttttatcttatttactttacgaaa

SEQ ID NO: 9 - DNA, 258 bp, Pichia pastoris
tgtgtctgtaaatttaaatccaaagaaaaataaagggcactacatagaacaacacaatcaacctacatagctctctttttttttttttttttttttttcttttttgttttttctcaattttcttcattttttgcattgttactactctcccattaagggaaattctaccaggaaaaccgaagaagacaaatgcaaaagggaaatatgaatacgcatgtatgcgcgcaaaaccgcacttacagagggcattaggacatt

SEQ ID NO: 10 - DNA, 552 bp, Pichia pastoris
agcaatgatataaacaacaattgagtgacaggtctactttgttctcaaaaggccataaccatctgtttgcatctcttatcaccacaccatcctcctcatctggccttcaattgtggggaacaactagcatcccaacaccagactaactccacccagatgaaaccagttgtcgcttaccagtcaatgaatgttgagctaacgttccttgaaactcgaatgatcccagccttgctgcgtatcatccctccgctattccgccgcttgctccaaccatgtttccgcctttttcgaacaagttcaaatacctatctttggcaggacttttcctcctgccttttttagcctcaggtctcggttagcctctaggcaaattctggtcttcatacctatatcaacttttcatcagatagcctttgggttcaaaaaagaactaaagcaggatgcctgatatataaatcccagatgatctgcttttgaaactattttcagtatcttgattcgtttacttacaaacaactattgttgattttatctggagaataatcgaacaaa

SEQ ID NO: 11 - DNA, 1102 bp, Pichia pastoris
cataatgatatttgagggtgttagttacttcgtctccagagtagcttatagggagaaaaaccgagacaacgatggaactcccatgtagattccaccgccccaattactgttttgggcaatcctgttgataagacgcattctagagttgtttcatgaaagggttacgggtgttgattggtttgagatatgccagaggacagatcaatctgtggtttgctaaactggaagtctggtaaggactctagcaagtccgttactcaaaaagtcataccaagtaagattacgtaacacctgggcatgactttctaagttagcaagtcaccaagagggtcctatttaacgtttggcggtatctgaaacacaagacttgcctatcccatagtacatcatattacctgtcaagctatgctaccccacagaaataccccaaaagttgaagtgaaaaaatgaaaattactggtaacttcaccccataacaaacttaataatttctgtagccaatgaaagtaaaccccattcaatgttccgagatttagtatacttgcccctataagaaacgaaggatttcagcttccttaccccatgaacagaaatcttccatttaccccccactggagagatccgcccaaacgaacagataatagaaaaaagaaattcggacaaatagaacactttctcagccaattaaagtcattccatgcactccctttagctgccgttccatccctttgttgagcaacaccatcgttagccagtacgaaagaggaaacttaaccgataccttggagaaatctaaggcgcgaatgagtttagcctagatatccttagtgaagggttgttccgatacttctccacattcagtcatagatgggcagctttgttatcatgaagagacggaaacgggcattaagggttaaccgccaaattatataaagacaacatgtccccagtttaaagtttttctttcctattcttgtatcctgagtgaccgttgtgtttaatataacaagttcgttttaacttaagaccaaaaccagttacaacaaattataacccctctaaacactaaagttcactcttatcaaactatcaaacatcaaaa

SEQ ID NO: 12 - DNA, 358 bp, Pichia pastoris
tgagataacagagttgggtaactagagagaataatagacgtatgcatgattactacacaacggatgtcgcactctttccttagttaaaactatcatccaatcacaagatgcgggctggaaagacttgctcccgaaggataatcttctgcttctatctcccttcctcatatggtttcgcagggctcatgccccttcttccttcgaactgcccgatgaggaagtccttagcctatcaaagaattcgggaccatcatcgatttttagagccttacctgatcgcaatcaggatttcactactcatataaatacatcgctcaaagctccaactttgcttgttcatacaattcttgatattcac

SEQ ID NO: 13 - DNA, 6688 bp, artificial
  Plasmid promoter sequence
attctggcccttgcacctgatcgcgaaggtggaaatggcagaaggatcagcctggacgaagcaaccagttccaactgctaagtaaagaagatgctagacgaaggagacttcagaggtgaaaagtttgcaagaagagagctgcgggaaataaattttcaatttaaggacttgagtgcgtccatattcgtgtacgtgtccaactgttttccattacctaagaaaaacataaagattaaaaagataaacccaatcgggaaactttagcgtgccgtttcggattccgaaaaacttttggagcgccagatgactatggaaagaggagtgtaccaaaatggcaagtcgggggctactcaccggatagccaatacattctctaggaaccagggatgaatccaggtttttgttgtcacggtaggtcaagcattcacttcttaggaatatctcgttgaaagctacttgaaatcccattgggtgcggaaccagcttctaattaaatagttcgatgatgttctctaagtgggactctacggctcaaacttctacacagcatcatcttagtagtcccttcccaaaacaccattctaggtttcggaacgtaacgaaacaatgttcctctcttcacattgggccgttactctagccttccgaagaaccaataaaagggaccggctgaaacgggtgtggaaactcctgtccagtttatggcaaaggctacagaaatcccaatcttgtcgggatgttgctcctcccaaacgccatattgtactgcagttggtgcgcattttagggaaaatttaccccagatgtcctgattttcgagggctacccccaactccctgtgcttatacttagtctaattctattcagtgtgctgacctacacgtaatgatgtcgtaacccagttaaatggccgaaaaactatttaagtaagtttatttctcctccagatgagactctccttcttttctccgctagttatcaaactataaacctattttacctcaaatacctccaacatcacccacttaaacacggccgaattcataatgagatttccttcaatttttactgcagttttattcgcagcatcctccgcattagctgctccagtcaacactacaacagaagatgaaacggcacaaattccggctgaagctgtcatcggttactcagatttagaaggggatttcgatgttgctgttttgccattttccaacagcacaaataacgggttattgtttataaatactactattgccagcattgctgctaaagaagaaggggtatctctcgagaaaagagaggctgaagctttaattaactgggccgcgaattaattcgccttagacatgactgttcctcagttcaagttgggcacttacgagaagaccggtcttgctagattctaatcaagaggatgtcagaatgccatttgcctgagagatgcaggcttcatttttgatacttttttatttgtaacctatatagtataggattttttttgtcattttgtttcttctcgtacgagcttgctcctgatcagcctatctcgcagctgatgaatatcttgtggtaggggtttgggaaaatcattcgagtttgatgtttttcttggtatttcccactcctcttcagagtacagaagattaagtgagacgttcgtttgtgcaagcttatcgataagctttaatgcggtagtttatcacagttaaattgctaacgcagtcaggcaccgtgtatgaaatctaacaatgcgctcatcgtcatcctcggcaccgtcaccctggatgctgtaggcataggcttggttatgccggtactgccgggcctcttgcgggatatcgtccattccgacagcatcgccagtcactatggcgtgctgctaggtacaacttgagcaagttgtcgatcagctcctcaaattggtcctctgtaacggatgactcaacttgcacattaacttgaagctcagtcgattgagtgaacttgatcaggttgtgcagctggtcagcagcatagggaaacacggcttttcctaccaaactcaaggaattatcaaactctgcaacacttgcgtatgcaggtagcaagggaaatgtcatacttgaagtcggacagtgagtgtagtcttgagaaattctgaagccgtatttttattatcagtgagtcagtcatcaggagatcctctacgccggacgcatcgtggccgacctgcagggggggggggggcgctgaggtctgcctcgtgaagaaggtgttgctgactcataccagctgaatcgccccatcatccagccagaaagtgagggagccacggttgatgagagctttgttgtaggtggaccagttggtgattttgaacttttgctttgccacggaacggtctgcgttgtcgggaagatgcgtgatctgatccttcaactcagcaaaagttcgatttattcaacaaagccgccgtcccgtcaagtcagcgtaatgctctgccagtgttacaaccaattaaccaattctgattagaaaaactcatcgagcatcaaatgaaactgcaatttattcatatcaggattatcaataccatatttttgaaaaagccgtttctgtaatgaaggagaaaactcaccgaggcagttccataggatggcaagatcctggtatcggtctgcgattccgactcgtccaacatcaatacaacctattaatttcccctcgtcaaaaataaggttatcaagtgagaaatcaccatgagtgacgactgaatccggtgagaatggcaaaagcttatgcatttctttccagacttgttcaacaggccagccattacgctcgtcatcaaaatcactcgcatcaaccaaaccgttattcattcgtgattgcgcctgagcgagacgaaatacgcgatcgctgttaaaaggacaattacaaacaggaatcgaatgcaaccggcgcaggaacactgccagcgcatcaacaatattttcacctgaatcaggatattcttctaatacctggaatgctgttttcccggggatcgcagtggtgagtaaccatgcatcatcaggagtacggataaaatgcttgatggtcggaagaggcataaattccgtcagccagtttagtctgaccatctcatctgtaacatcattggcaacgctacctttgccatgtttcagaaacaactctggcgcatcgggcttcccatacaatcgatagattgtcgcacctgattgcccgacattatcgcgagcccatttatacccatataaatcagcatccatgttggaatttaatcgcggcctcgagcaagacgtttcccgttgaatatggctcataacaccccttgtattactgtttatgtaagcagacagttttattgttcatgatgatatatttttatcttgtgcaatgtaacatcagagattttgagacacaacgtggctttcccccccccccctgcaggtcggcatcaccggcgccacaggtgcggttgctggcgcctatatcgccgacatcaccgatggggaagatcgggctcgccacttcgggctcatgagcgcttgtttcggcgtgggtatggtggcaggccccgtggccgggggactgttgggcgccatctccttgcatgcaccattccttgcggcggcggtgctcaacggcctcaacctactactgggctgcttcctaatgcaggagtcgcataagggagagcgtcgagtatctatgattggaagtatgggaatggtgatacccgcattcttcagtgtcttgaggtctcctatcagattatgcccaactaaagcaaccggaggaggagatttcatggtaaatttctctgacttttggtcatcagtagactcgaactgtgagactatctcggttatgacagcagaaatgtccttcttggagacagtaaatgaagtcccaccaataaagaaatccttgttatcaggaacaaacttcttgtttcgaactttttcggtgccttgaactataaaatgtagagtggatatgtcgggtaggaatggagcgggcaaatgcttaccttctggaccttcaagaggtatgtagggtttgtagatactgatgccaacttcagtgacaacgttgctatttcgttcaaaccattccgaatccagagaaatcaaagttgtttgtctactattgatccaagccagtgcggtcttgaaactgacaatagtgtgctcgtgttttgaggtcatctttgtatgaataaatctagtctttgatctaaataatcttgacgagccaaggcgataaatacccaaatctaaaactcttttaaaacgttaaaaggacaagtatgtctgcctgtattaaaccccaaatcagctcgtagtctgatcctcatcaacttgaggggcactatcttgttttagagaaatttgcggagatgcgatatcgagaaaaaggtacgctgattttaaacgtgaaatttatctcaagatctctgcctcgcgcgtttcggtgatgacggtgaaaacctctgacacatgcagctcccggagacggtcacagcttgtctgtaagcggatgccgggagcagacaagcccgtcagggcgcgtcagcgggtgttggcgggtgtcggggcgcagccatgacccagtcacgtagcgatagcggagtgtatactggcttaactatgcggcatcagagcagattgtactgagagtgcaccatatgcggtgtgaaataccgcacagatgcgtaaggagaaaataccgcatcaggcgctcttccgcttcctcgctcactgactcgctgcgctcggtcgttcggctgcggcgagcggtatcagctcactcaaaggcggtaatacggttatccacagaatcaggggataacgcaggaaagaacatgtgagcaaaaggccagcaaaaggccaggaaccgtaaaaaggccgcgttgctggcgtttttccataggctccgcccccctgacgagcatcacaaaaatcgacgctcaagtcagaggtggcgaaacccgacaggactataaagataccaggcgtttccccctggaagctccctcgtgcgctctcctgttccgaccctgccgcttaccggatacctgtccgcctttctcccttcgggaagcgtggcgctttctcaatgctcacgctgtaggtatctcagttcggtgtaggtcgttcgctccaagctgggctgtgtgcacgaaccccccgttcagcccgaccgctgcgccttatccggtaactatcgtcttgagtccaacccggtaagacacgacttatcgccactggcagcagccactggtaacaggattagcagagcgaggtatgtaggcggtgctacagagttcttgaagtggtggcctaactacggctacactagaaggacagtatttggtatctgcgctctgctgaagccagttaccttcggaaaaagagttggtagctcttgatccggcaaacaaaccaccgctggtagcggtggtttttttgtttgcaagcagcagattacgcgcagaaaaaaaggatctcaagaagatcctttgatcttttctacggggtctgacgctcagtggaacgaaaactcacgttaagggattttggtcatgagattatcaaaaaggatcttcacctagatccttttaaattaaaaatgaagttttaaatcaatctaaagtatatatgagtaaacttggtctgacagttaccaatgcttaatcagtgaggcacctatctcagcgatctgtctatttcgttcatccatagttgcctgactccccgtcgtgtagataactacgatacgggagggcttaccatctggccccagtgctgcaatgataccgcgagacccacgctcaccggctccagatttatcagcaataaaccagccagccggaagggccgagcgcagaagtggtcctgcaactttatccgcctccatccagtctattaattgttgccgggaagctagagtaagtagttcgccagttaatagtttgcgcaacgttgttgccattgctgcaggcatcgtggtgtcacgctcgtcgtttggtatggcttcattcagctccggttcccaacgatcaaggcgagttacatgatcccccatgttgtgcaaaaaagcggttagctccttcggtcctccgatcgttgtcagaagtaagttggccgcagtgttatcactcatggttatggcagcactgcataattctcttactgtcatgccatccgtaagatgcttttctgtgactggtgagtactcaaccaagtcattctgagaatagtgtatgcggcgaccgagttgctcttgcccggcgtcaacacgggataataccgcgccacatagcagaactttaaaagtgctcatcattggaaaacgttcttcggggcgaaaactctcaaggatcttaccgctgttgagatccagttcgatgtaacccactcgtgcacccaactgatcttcagcatcttttactttcaccagcgtttctgggtgagcaaaaacaggaaggcaaaatgccgcaaaaaagggaataagggcgacacggaaatgttgaatactcatactcttcctttttcaatattattgaagcatttatcagggttattgtctcatgagcggatacatatttgaatgtatttagaaaaataaacaaataggggttccgcgcacatttccccgaaaagtgccacctgacgtc

SEQ ID NO: 14 - DNA, 159 bp, human
aatagtgactctgaatgccctttgtcccatgacggatactgtcttcacgacggcgtttgtatgtatatcgaggcactagataagtatgcatgtaactgcgtagtaggatacattggagaacgttgccaataccgtgatttgaagtggtgggagttgcgt

SEQ ID NO: 15 - DNA, 666 bp, human
tggacgggcgaggactcggcggagcccaactctgactcggcggagtggatccgagacatgtacgccaaggtcacggagatctggcaggaggtcatgcagcggcgggacgacgacggcgcgctccacgccgcctgccaggtgcagccgtcggccacgctggacgccgcgcagccccgggtgaccggcgtcgtcctcttccggcagcttgcgccccgcgccaagctcgacgccttcttcgccctggagggcttcccgaccgagccgaacagctccagccgcgccatccacgtgcaccagttcggggacctgagccagggctgcgagtccaccgggccccactacaacccgctggccgtgccgcacccgcagcacccgggcgacttcggcaacttcgcggtccgcgacggcagcctctggaggtaccgcgccggcctggccgcctcgctcgcgggcccgcactccatcgtgggccgggccgtggtcgtccacgctggcgaggacgacctgggccgcggcggtaaccaggccagcgtggagaacgggaacgcgggccggcggctggcctgctgcgtggtgggcgtgtgcgggcccgggctctgggagcgccaggcgcgggagcactcagagcgcaagaagcggcggcgcgagagcgagtgcaaggccgcc

SEQ ID NO: 16 - DNA, 2076 bp, human
ggccgtaggagaaggagtgttcagtggtgcgccgtatcccaacccgaggccacaaaatgcttccaatggcaaaggaatatgagaaaagtgcgtggccctcctgtcagctgcataaagagagactcccccatccagtgtatccaggccattgcggaaaacagggccgatgctgtgacccttgatggtggtttcatatacgaggcaggcctggccccctacaaactgcgacctgtagcggcggaagtctacgggaccgaaagacagccacgaactcactattatgccgtggctgtggtgaagaagggcggcagctttcagctgaacgaactgcaaggtctgaagtcctgccacacaggccttcgcaggaccgctggatggaatgtccctatagggacacttcgtccattcttgaattggacgggtccacctgagcccattgaggcagctgtggccaggttcttctcagccagctgtgttcccggtgcagataaaggacagttccccaacctgtgtcgcctgtgtgcggggacaggggaaaacaaatgtgccttctcctcccaggaaccgtacttcagctactctggtgccttcaagtgtctgagagacggggctggagacgtggcttttatcagagagagcacagtgtttgaggacctgtcagacgaggctgaaagggacgagtatgagttactctgcccagacaacactcggaagccagtggacaagttcaaagactgccatctggcccgggtcccttctcatgccgttgtggcacgaagtgtgaatggcaaggaggatgccatctggaatcttctccgccaggcacaggaaaagtttggaaaggacaagtcaccgaaattccagctctttggctcccctagtgggcagaaagatctgctgttcaaggactctgccattgggttttcgagggtgcccccgaggatagattctgggctgtaccttggctccggctacttcactgccatccagaacttgaggaaaagtgaggaggaagtggctgcccggcgtgcgcgggtcgtgtggtgtgcggtgggcgagcaggagctgcgcaagtgtaaccagtggagtggcttgagcgaaggcagcgtgacctgctcctcggcctccaccacagaggactgcatcgccctggtgctgaaaggagaagctgatgccatgagtttggatggaggatatgtgtacactgcaggcaaatgtggtttggtgcctgtcctggcagagaactacaaatcccaacaaagcagtgaccctgatcctaactgtgtggatagacctgtggaaggatatcttgctgtggcggtggttaggagatcagacactagccttacctggaactctgtgaaaggcaagaagtcctgccacaccgccgtggacaggactgcaggctggaatatccccatgggcctgctcttcaaccagacgggctcctgcaaatttgatgaatatttcagtcaaagctgtgcccctgggtctgacccgagatctaatctctgtgctctgtgtattggcgacgagcagggtgagaataagtgcgtgcccaacagcaacgagagatactacggctacactggggctttccggtgcctggctgagaatgctggagacgttgcatttgtgaaagatgtcactgtcttgcagaacactgatggaaataacaatgaggcatgggctaaggatttgaagctggcagactttgcgctgctgtgcctcgatggcaaacggaagcctgtgactgaggctagaagctgccatcttgccatggccccgaatcatgccgtggtgtctcggatggataaggtggaacgcctgaaacaggtgttgctccaccaacaggctaaatttgggagaaatggatctgactgcccggacaagttttgcttattccagtctgaaaccaaaaaccttctgttcaatgacaacactgagtgtctggccagactccatggcaaaacaacatatgaaaaatatttgggaccacagtatgtcgcaggcattactaatctgaaaaagtgctcaacctcccccctcctggaagcctgtgagttcctcaggaag

SEQ ID NO: 17 - protein, 53 aa, human
NSDSECPLSHDGYCLHDGVCMYIEALDKYACNCVVGYIGERCQYRDLKWWELR

SEQ ID NO: 18 - protein, 222 aa, human
WTGEDSAEPNSDSAEWIRDMYAKVTEIWQEVMQRRDDDGALHAACQVQPSATLDAAQPRVTGVVLFRQLAPRAKLDAFFALEGFPTEPNSSSRAIHVHQFGDLSQGCESTGPHYNPLAVPHPQHPGDFGNFAVRDGSLWRYRAGLAASLAGPHSIVGRAVVVHAGEDDLGRGGNQASVENGNAGRRLACCVVGVCGPGLWERQAREHSERKKRRRESECKAA

SEQ ID NO: 19 - protein, 692 aa, human
GRRRRSVQWCAVSQPEATKCFQWQRNMRKVRGPPVSCIKRDSPIQCIQAIAENRADAVTLDGGFIYEAGLAPYKLRPVAAEVYGTERQPRTHYYAVAVVKKGGSFQLNELQGLKSCHTGLRRTAGWNVPIGTLRPFLNWTGPPEPIEAAVARFFSASCVPGADKGQFPNLCRLCAGTGENKCAFSSQEPYFSYSGAFKCLRDGAGDVAFIRESTVFEDLSDEAERDEYELLCPDNTRKPVDKFKDCHLARVPSHAVVARSVNGKEDAIWNLLRQAQEKFGKDKSPKFQLFGSPSGQKDLLFKDSAIGFSRVPPRIDSGLYLGSGYFTAIQNLRKSEEEVAARRARVVWCAVGEQELRKCNQWSGLSEGSVTCSSASTTEDCIALVLKGEADAMSLDGGYVYTAGKCGLVPVLAENYKSQQSSDPDPNCVDRPVEGYLAVAVVRRSDTSLTWNSVKGKKSCHTAVDRTAGWNIPMGLLFNQTGSCKFDEYFSQSCAPGSDPRSNLCALCIGDEQGENKCVPNSNERYYGYTGAFRCLAENAGDVAFVKDVTVLQNTDGNNNEAWAKDLKLADFALLCLDGKRKPVTEARSCHLAMAPNHAVVSRMDKVERLKQVLLHQQAKFGRNGSDCPDKFCLFQSETKNLLFNDNTECLARLHGKTTYEKYLGPQYVAGITNLKKCSTSPLLEACEFLRK

SEQ ID NO: 20 - DNA, 651 bp, SARS-CoV-2
gtacagcctacagaaagtattgtccgtttccctaatatcaccaatttatgcccttttggtgaagtcttcaatgccaccagattcgcctccgtatatgcctggaaccgtaagagaatcagtaattgcgtggccgattattctgtgttgtataatagtgcctccttctccaccttcaagtgttatggcgtgtcccctactaagctgaatgacttatgttttaccaatgtttatgcagactcattcgtcatccgtggagatgaagtccgtcaaattgcccccggacagacaggaaaaatcgccgactataattataaactgcctgatgacttcaccggatgtgtcatcgcatggaatagtaataatttagattcaaaagtaggaggaaattataattatctttaccgtctgtttagaaaatcaaacttgaaaccattcgagagagatatttccacagagatctaccaggcaggatccaccccttgcaatggagtcgaaggattcaattgctattttcctctgcagtcttatggatttcagcctacaaatggagtcggataccaaccttatagagtcgtggtcttaagtttcgagttgcttcacgccgtcgccacagtgtgcggacctaaaaagtcaacaaatttagtcaagaat

SEQ ID NO: 21 - protein, 217 aa, SARS-CoV-2
VQPTESIVRFPNITNLCPFGEVFNATRFASVYAWNRKRISNCVADYSVLYNSASFSTFKCYGVSPTKLNDLCFTNVYADSFVIRGDEVRQIAPGQTGKIADYNYKLPDDFTGCVIAWNSNNLDSKVGGNYNYLYRLFRKSNLKPFERDISTEIYQAGSTPCNGVEGFNCYFPLQSYGFQPTNGVGYQPYRVVVLSFELLHAVATVCGPKKSTNLVKN